European Patent Application EP 4 502 181 A1, published February 5, 2025. Title: IFI16 Mutant Gene as a Marker for Risk Prediction, Diagnosis or Prognosis of Chronic Liver Disease and Uses Thereof. Applicant: NATIONAL CANCER CENTER. The sequence listing filed with the application follows.

SEQUENCE LISTING (14 sequences)

SEQ ID NO: 1 - DNA, 501 bp, Homo sapiens
  source 1..501: mol_type = genomic DNA
ttctctggggcaatagcagaataggagcaagccagcactagtcagctaactaagtgactcaaccaaggccttttttccttgttatctttgcagatacttcattttcttagcgtttctggagattacaacatcctgcggttccgtttctgggaactttactgatttatctcccccctcacacaaataagcattgattcctgcatttctgaagatctcaagatctggactactgttgaaaaaatttccagtgaggtgagtactgttcctgattttgtaaatatgatcttgttccttccttgaagtccccagaatcacaaggggacaatcagtattggttattcagggtcatgggatgatgggagtagggctgagtattcagaaaagtgaaaactgagttgcttgatatgaatccttcatttacttaggaagataacaggcatcttctattccaccacaactgaggactgaacaagagaaaatgcattttgaccgttgcagatt

SEQ ID NO: 2 - DNA, 601 bp, Homo sapiens
  source 1..601: mol_type = genomic DNA
ctctgccctcctgaaagttaatgattttttttttccttgtggcaaggtataggggagtggaggggaaggcagttaggaaaaggttactattgtttacttttcaaatttttaaaagatgttttctatagcctggtacaatatttcatgtgtgcttaaatggaatgtgagattcttaaatgttgttttcagaattttattagataaatgttgttaattacgttgttcaaatttattatatcattacagattttttcaccttgttcatttagtaattgaagcataaactgaaatctcctattataaagtttgcttttttggccgggcacagaggttcatgcctgtaatcccagtactttgggggagaccaaggcgagcggatcacttgacgtcaggagttccagaccagcctggccagcatggcgaaaccctgtctctattaaaaatacaataattagccgggtatggtcatgtgtgcctgtaatcccagctactcaggagactgaggcaggagaatcgcttgaaccaggaggcagaggttgcagtgagccgagactgtgccactacactccagcctgggtgacagagcaaggctctgtctcaa

SEQ ID NO: 3 - DNA, 501 bp, Homo sapiens
  source 1..501: mol_type = genomic DNA
catgctctcagattgctccagttctcaggaccagcagtcaaacatttcaaaccttctttgatagcaattgcaccaggaataccttttgtactctcccccttccttctgcccaatgaaaaccctctcctcaactcttgtcattgggtgcaccagctcctttctctctcctgttgttccctgacatctcctgctctttcacttgcactcatgctgagtaggagtgaatatctcatttcacggtccaaattaaacagagaggcatgactcaaaggtcaagaatttattaagggagatagatgagagcgagaaaagaatcatttagaaaggaataggggaagagatatggtgcagggggaggagatacagtgtgattgaagggagaaatgtaggatcatcagcatctcaactggtctgtctttatctctttctccttcaaggtcatcaagaccaggaaaaacaagaaagacatactcaatcctgattcaagtatggaaacttcac

SEQ ID NO: 4 - DNA, 501 bp, Homo sapiens
  source 1..501: mol_type = genomic DNA
aattaaacagagaggcatgactcaaaggtcaagaatttattaagggagatagatgagagcgagaaaagaatcatttagaaaggaataggggaagagatatggtgcagggggaggagatacagtgtgattgaagggagaaatgtaggatcatcagcatctcaactggtctgtctttatctctttctccttcaaggtcatcaagaccaggaaaaacaagaaagacatactcaatcctgattcaagtatggaaacttcaccagactttttcttctaaaatctggatgtcattgacgataatgtttatggagataaggtctaagtgcctaaaaaaatgtacatatacctggttgaaatacaacactatacatacacaccaccatatatactagctgttaatcctatggaatggggtattgggagtgcttttttaatttttcatagtttttttttaataaaatggcatattttgcatctacaacttctataatttgaaaaaataaa

SEQ ID NO: 5 - DNA, 21 bp, synthetic construct
  source 1..21: mol_type = other DNA
gggcaatagcagaataggagc

SEQ ID NO: 6 - DNA, 23 bp, synthetic construct
  source 1..23: mol_type = other DNA
tctcttgttcagtcctcagttgt

SEQ ID NO: 7 - DNA, 20 bp, synthetic construct
  source 1..20: mol_type = other DNA
tggcaaggtataggggagtg

SEQ ID NO: 8 - DNA, 20 bp, synthetic construct
  source 1..20: mol_type = other DNA
gctggagtgtagtggcacag

SEQ ID NO: 9 - DNA, 21 bp, synthetic construct
  source 1..21: mol_type = other DNA
catgctctcagattgctccag

SEQ ID NO: 10 - DNA, 22 bp, synthetic construct
  source 1..22: mol_type = other DNA
tttcctggtcttgatgaccttg

SEQ ID NO: 11 - DNA, 19 bp, synthetic construct
  source 1..19: mol_type = other DNA
gcagggggaggagatacag

SEQ ID NO: 12 - DNA, 22 bp, synthetic construct
  source 1..22: mol_type = other DNA
cccattccataggattaacagc

SEQ ID NO: 13 - protein, 785 aa, Homo sapiens
MGKKYKNIVLLKGLEVINDYHFRMVKSLLSNDLKLNLKMREEYDKIQIADLMEEKFRGDAGLGKLIKIFEDIPTLEDLAETLKKEKLKVKGPALSRKRKKEVDATSPAPSTSSTVKTEGAEATPGAQKRKKSTKEKAGPKGSKVSEEQTQPPSPAGAGMSTAMGRSPSPKTSLSAPPNSSSTENPKTVAKCQVTPRRNVLQKRPVIVKVLSTTKPFEYETPEMEKKIMFHATVATQTQFFHVKVLNTSLKEKFNGKKIIIISDYLEYDSLLEVNEESTVSEAGPNQTFEVPNKIINRAKETLKIDILHKQASGNIVYGVFMLHKKTVNQKTTIYEIQDDRGKMDVVGTGQCHNIPCEEGDKLQLFCFRLRKKNQMSKLISEMHSFIQIKKKTNPRNNDPKSMKLPQEQRQLPYPSEASTTFPESHLRTPQMPPTTPSSSFFTKKSEDTISKMNDFMRMQILKEGSHFPGPFMTSIGPAESHPHTPQMPPSTPSSSFLTTKSEDTISKMNDFMRMQILKEGSHFPGPFMTSIGPAESHPHTPQMPPSTPSSSFLTTLKPRLKTEPEEVSIEDSAQSDLKEVMVLNATESFVYEPKEQKKMFHATVATENEVFRVKVFNIDLKEKFTPKKIIAIANYVCRNGFLEVYPFTLVADVNADRNMEIPKGLIRSASVTPKINQLCSQTKGSFVNGVFEVHKKNVRGEFTYYEIQDNTGKMEVVVHGRLTTINCEEGDKLKLTCFELAPKSGNTGELRSVIHSHIKVIKTRKNKKDILNPDSSMETSPDFFF

SEQ ID NO: 14 - protein, 785 aa, Homo sapiens
MGKKYKNIVLLKGLEVINDYHFRMVKSLLSNDLKLNLKMREEYDKIQIADLMEEKFRGDAGLGKLIKIFEDIPTLEDLAETLKKEKLKVKGPALSRKRKKEVDATSPAPSTSSTVKTEGAEATPGAQKRKKSTKEKAGPKGSKVSEEQTQPPSPAGAGMSTAMGRSPSPKTSLSAPPNSSSTENPKTVAKCQVTPRRNVLQKRPVIVKVLSTTKPFEYETPEMEKKIMFHATVATQTQFFHVKVLNTSLKEKFNGKKIIIISDYLEYDSLLEVNEESTVSEAGPNQTFEVPNKIINRAKETLKIDILHKQASGNIVYGVFMLHKKTVNQKTTIYEIQDDRGKMDVVGTGQCHNIPCEEGDKLQLFCFRLRKKNQMSKLISEMHSFIQIKKKTNPRNNDPKSMKLPQEQRQLPYPSEASTTFPESHLRTPQMPPTTPSSSFFTKKSEDTISKMNDFMRMQILKEGSHFPGPFMTSIGPAESHPHTPQMPPSTPSSSFLTTKSEDTISKMNDFMRMQILKEGSHFPGPFMTSIGPAESHPHTPQMPPSTPSSSFLTTLKPRLKTEPEEVSIEDSAQSDLKEVMVLNATESFVYEPKEQKKMFHATVATENEVFRVKVFNIDLKEKFTPKKIIAIANYVCRNGFLEVYPFTLVADVNADRNMEIPKGLIRSASVTPKINQLCSQTKGSFVNGVFEVHKKNVRGEFTYYEIQDNTGKMEVVVHGRLSTINCEEGDKLKLTCFELAPKSGNTGELRSVIHSHIKVIKTRKNKKDILNPDSSMETSPDFFF